European Patent Application EP 4 744 731 A2, published May 20, 2026. Title: ANTI-HUMAN P40 PROTEIN DOMAIN ANTIBODY AND USE THEREOF. Applicant: Akeso Biopharma, Inc. Application EP, filed July 28, 2020. The sequence listing filed with the application follows.

SEQUENCE LISTING (54 sequences)

SEQ ID NO: 1 - protein, 119 aa, synthetic construct
  REGION 1..119: note = Artificially Synthesized Sequence
EVQLVQSGAEVKKPGESLKISCQSSGYSFTTYWIGWVRQMPGQGLEWIGIMSPVDSDIRYNPMFRGQVTMSVDKSSSTAYLQWSSLKASDTAMYYCARRRPGQGYFDFWGQGTMVTVSS

SEQ ID NO: 2 - DNA, 357 bp, synthetic construct
  misc_feature 1..357: note = Artificially Synthesized Sequence
  source 1..357: mol_type = other DNA
gaggtgcagctggtgcagtctggggccgaagtgaagaaacccggggagagtctgaagatctcatgccagagctccggctactccttcaccacatattggatcgggtgggtgagacagatgcctggccaggggctggaatggatcggaattatgagcccagtggactccgatattcgctacaaccccatgtttcgaggccaggtgacaatgagcgtggacaagtctagttcaactgcttatctgcagtggagctccctgaaagccagcgataccgctatgtactattgtgcccggagaaggcctggacagggctacttcgacttttgggggcagggaactatggtgaccgtctctagt

SEQ ID NO: 3 - protein, 8 aa, synthetic construct
  REGION 1..8: note = Artificially Synthesized Sequence
GYSFTTYW

SEQ ID NO: 4 - protein, 8 aa, synthetic construct
  REGION 1..8: note = Artificially Synthesized Sequence
MSPVDSDI

SEQ ID NO: 5 - protein, 12 aa, synthetic construct
  REGION 1..12: note = Artificially Synthesized Sequence
ARRRPGQGYFDF

SEQ ID NO: 6 - protein, 107 aa, synthetic construct
  REGION 1..107: note = Artificially Synthesized Sequence
DIQMTQSPSSLSASVGDRVTITCKASQNVGSWLAWYQQKPGKAPKSLIYSASSRQSGVPSRFSGSGSGTDFTLTISSLQPEDFATYYCQQYDIYPFTFGQGTKLEIK

SEQ ID NO: 7 - DNA, 321 bp, synthetic construct
  misc_feature 1..321: note = Artificially Synthesized Sequence
  source 1..321: mol_type = other DNA
gatattcagatgacccagagcccttcaagcctgtccgcaagcgtcggggatagagtgaccattacctgtaaagcaagccagaacgtgggaagctggctggcctggtaccagcagaagccaggcaaagcacccaagtctctgatctatagtgcaagctcccggcagtcaggagtgccaagcagattcagtggctcagggagcggaacagactttaccctgacaatctctagtctgcagcctgaggacttcgcaacttactattgccagcagtacgatatctacccattcacatttggccaggggactaaactggagatcaag

SEQ ID NO: 8 - protein, 6 aa, synthetic construct
  REGION 1..6: note = Artificially Synthesized Sequence
QNVGSW

SEQ ID NO: 9 - skipped

SEQ ID NO: 10 - protein, 9 aa, synthetic construct
  REGION 1..9: note = Artificially Synthesized Sequence
QQYDIYPFT

SEQ ID NO: 11 - protein, 107 aa, synthetic construct
  REGION 1..107: note = Artificially Synthesized Sequence
EIVLTQSPATLSASPGERATISCRASQSVGSWLAWYQQKPGQAPRSLIYAASNLQSGIPARFSGSGSGTDFTLTISSLEPEDFAVYYCQQYNIYPYTFGQGTRLEIK

SEQ ID NO: 12 - DNA, 321 bp, synthetic construct
  misc_feature 1..321: note = Artificially Synthesized Sequence
  source 1..321: mol_type = other DNA
gagatcgtcctgacacagagtcctgctaccctgagcgcttccccaggagagagggcaaccatctcctgccgcgcctctcagagcgttggctcctggctggcttggtaccagcagaagccaggccaggcaccccgaagcctgatctatgccgcttctaatctgcagagcgggattcccgctagattctctggcagtgggtcaggaacagactttaccctgacaatctcaagcctggagcctgaagatttcgccgtgtactattgccagcagtacaacatctacccatatacatttggccaggggactcggctggagatcaag

SEQ ID NO: 13 - protein, 107 aa, synthetic construct
  REGION 1..107: note = Artificially Synthesized Sequence
EIVLTQSPATLSASPGERATISCRASQSVSSWLAWYQQKPGQAPRSLIYSASNLQSGIPARFSGSGSGTDFTLTISSLEPEDFAVYYCQQYNIYPYTFGQGTRLEIK

SEQ ID NO: 14 - DNA, 321 bp, synthetic construct
  misc_feature 1..321: note = Artificially Synthesized Sequence
  source 1..321: mol_type = other DNA
gagatcgtcctgacacagagtcctgctaccctgagcgcttccccaggagagagggcaaccatctcctgccgcgcctctcagagcgttagctcctggctggcttggtaccagcagaagccaggccaggcaccccgaagcctgatctattccgcttctaatctgcagagcgggattcccgctagattctctggcagtgggtcaggaacagactttaccctgacaatctcaagcctggagcctgaagatttcgccgtgtactattgccagcagtacaacatctacccatatacatttggccaggggactcggctggagatcaag

SEQ ID NO: 15 - protein, 107 aa, synthetic construct
  REGION 1..107: note = Artificially Synthesized Sequence
EIVLTQSPATLSASPGERATISCRASQSVSSWLAWYQQKPGQAPRSLIYAASNRQSGIPARFSGSGSGTDFTLTISSLEPEDFAVYYCQQYNIYPYTFGQGTRLEIK

SEQ ID NO: 16 - DNA, 321 bp, synthetic construct
  misc_feature 1..321: note = Artificially Synthesized Sequence
  source 1..321: mol_type = other DNA
gagatcgtcctgacacagagtcctgctaccctgagcgcttccccaggagagagggcaaccatctcctgccgcgcctctcagagcgttagctcctggctggcttggtaccagcagaagccaggccaggcaccccgaagcctgatctatgccgcttctaatcggcagagcgggattcccgctagattctctggcagtgggtcaggaacagactttaccctgacaatctcaagcctggagcctgaagatttcgccgtgtactattgccagcagtacaacatctacccatatacatttggccaggggactcggctggagatcaag

SEQ ID NO: 17 - protein, 107 aa, synthetic construct
  REGION 1..107: note = Artificially Synthesized Sequence
EIVLTQSPATLSASPGERATISCRASQSVSSWLAWYQQKPGQAPRSLIYAASNLQSGIPARFSGSGSGTDFTLTISSLEPEDFAVYYCQQYNIYPFTFGQGTRLEIK

SEQ ID NO: 18 - DNA, 321 bp, synthetic construct
  misc_feature 1..321: note = Artificially Synthesized Sequence
  source 1..321: mol_type = other DNA
gagatcgtcctgacacagagtcctgctaccctgagcgcttccccaggagagagggcaaccatctcctgccgcgcctctcagagcgttagctcctggctggcttggtaccagcagaagccaggccaggcaccccgaagcctgatctatgccgcttctaatctgcagagcgggattcccgctagattctctggcagtgggtcaggaacagactttaccctgacaatctcaagcctggagcctgaagatttcgccgtgtactattgccagcagtacaacatctacccatttacatttggccaggggactcggctggagatcaag

SEQ ID NO: 19 - protein, 6 aa, synthetic construct
  REGION 1..6: note = Artificially Synthesized Sequence
QSVGSW

SEQ ID NO: 20 - protein, 6 aa, synthetic construct
  REGION 1..6: note = Artificially Synthesized Sequence
QSVSSW

SEQ ID NO: 21 - skipped

SEQ ID NO: 22 - protein, 9 aa, synthetic construct
  REGION 1..9: note = Artificially Synthesized Sequence
QQYNIYPYT

SEQ ID NO: 23 - protein, 9 aa, synthetic construct
  REGION 1..9: note = Artificially Synthesized Sequence
QQYNIYPFT

SEQ ID NO: 24 - protein, 119 aa, synthetic construct
  REGION 1..119: note = Artificially Synthesized Sequence
EVQLVQSGAEVKKPGESLKISCQSSGYTFTSYWIGWVRQMPGQGLEWIGIMSPVDSDIRYNPMFRGQVTMSVDKSSSTAYLQWSSLKASDTAMYYCARRRPGQGYFDFWGQGTMVTVSS

SEQ ID NO: 25 - protein, 107 aa, synthetic construct
  REGION 1..107: note = Artificially Synthesized Sequence
EIVLTQSPATLSASPGERATISCRASQSVGTWVAWYQQKPGQAPRSLIYAASNLQSGIPARFSGSGSGTDFTLTISSLEPEDFAVYYCQQYNIYPYTFGQGTRLEIK

SEQ ID NO: 26 - protein, 8 aa, synthetic construct
  REGION 1..8: note = Artificially Synthesized Sequence
GYTFTSYW

SEQ ID NO: 27 - protein, 6 aa, synthetic construct
  REGION 1..6: note = Artificially Synthesized Sequence
QSVGTW

SEQ ID NO: 28 - skipped

SEQ ID NO: 29 - protein, 25 aa, synthetic construct
  REGION 1..25: note = Artificially Synthesized Sequence
EVQLVQSGAEVKKPGESLKISCQSS

SEQ ID NO: 30 - protein, 17 aa, synthetic construct
  REGION 1..17: note = Artificially Synthesized Sequence
IGWVRQMPGQGLEWIGI

SEQ ID NO: 31 - protein, 38 aa, synthetic construct
  REGION 1..38: note = Artificially Synthesized Sequence
RYNPMFRGQVTMSVDKSSSTAYLQWSSLKASDTAMYYC

SEQ ID NO: 32 - protein, 11 aa, synthetic construct
  REGION 1..11: note = Artificially Synthesized Sequence
WGQGTMVTVSS

SEQ ID NO: 33 - protein, 26 aa, synthetic construct
  REGION 1..26: note = Artificially Synthesized Sequence
EIVLTQSPATLSASPGERATISCRAS

SEQ ID NO: 34 - protein, 17 aa, synthetic construct
  REGION 1..17: note = Artificially Synthesized Sequence
VAWYQQKPGQAPRSLIY

SEQ ID NO: 35 - protein, 36 aa, synthetic construct
  REGION 1..36: note = Artificially Synthesized Sequence
NLQSGIPARFSGSGSGTDFTLTISSLEPEDFAVYYC

SEQ ID NO: 36 - protein, 10 aa, synthetic construct
  REGION 1..10: note = Artificially Synthesized Sequence
FGQGTRLEIK

SEQ ID NO: 37 - DNA, 357 bp, synthetic construct
  misc_feature 1..357: note = Artificially Synthesized Sequence
  source 1..357: mol_type = other DNA
gaggtgcagctggtgcagtctggggccgaagtgaagaaacccggggagagtctgaagatctcatgccagagctccggctacaccttcacctcatattggatcgggtgggtgagacagatgcctggccaggggctggaatggatcggaattatgagcccagtggactccgatattcgctacaaccccatgtttcgaggccaggtgacaatgagcgtggacaagtctagttcaactgcttatctgcagtggagctccctgaaagccagcgataccgctatgtactattgtgcccggagaaggcctggacagggctacttcgacttttgggggcagggaactatggtgaccgtctctagt

SEQ ID NO: 38 - DNA, 321 bp, synthetic construct
  misc_feature 1..321: note = Artificially Synthesized Sequence
  source 1..321: mol_type = other DNA
gagatcgtcctgacacagagtcctgctaccctgagcgcttccccaggagagagggcaaccatctcctgccgcgcctctcagagcgttggcacctgggtggcttggtaccagcagaagccaggccaggcaccccgaagcctgatctatgccgcttctaatctgcagagcgggattcccgctagattctctggcagtgggtcaggaacagactttaccctgacaatctcaagcctggagcctgaagatttcgccgtgtactattgccagcagtacaacatctacccatatacatttggccaggggactcggctggagatcaag

SEQ ID NO: 39 - protein, 449 aa, synthetic construct
  REGION 1..449: note = Artificially Synthesized Sequence
EVQLVQSGAEVKKPGESLKISCQSSGYTFTSYWIGWVRQMPGQGLEWIGIMSPVDSDIRYNPMFRGQVTMSVDKSSSTAYLQWSSLKASDTAMYYCARRRPGQGYFDFWGQGTMVTVSSASTKGPSVFPLAPSSKSTSGGTAALGCLVKDYFPEPVTVSWNSGALTSGVHTFPAVLQSSGLYSLSSVVTVPSSSLGTQTYICNVNHKPSNTKVDKKVEPKSCDKTHTCPPCPAPELLGGPSVFLFPPKPKDTLMISRTPEVTCVVVDVSHEDPEVKFNWYVDGVEVHNAKTKPREEQYNSTYRVVSVLTVLHQDWLNGKEYKCKVSNKALPAPIEKTISKAKGQPREPQVYTLPPSREEMTKNQVSLTCLVKGFYPSDIAVEWESNGQPENNYKTTPPVLDSDGSFFLYSKLTVDKSRWQQGNVFSCSVMHEALHNHYTQKSLSLSPGK

SEQ ID NO: 40 - protein, 214 aa, synthetic construct
  REGION 1..214: note = Artificially Synthesized Sequence
EIVLTQSPATLSASPGERATISCRASQSVGTWVAWYQQKPGQAPRSLIYAASNLQSGIPARFSGSGSGTDFTLTISSLEPEDFAVYYCQQYNIYPYTFGQGTRLEIKRTVAAPSVFIFPPSDEQLKSGTASVVCLLNNFYPREAKVQWKVDNALQSGNSQESVTEQDSKDSTYSLSSTLTLSKADYEKHKVYACEVTHQGLSSPVTKSFNRGEC

SEQ ID NO: 41 - protein, 26 aa, synthetic construct [sequence omitted]

SEQ ID NO: 42 - protein, 18 aa, synthetic construct
  REGION 1..18: note = Artificially Synthesized Sequence
LAWYQQKPGKAPKSLIYS

SEQ ID NO: 43 - protein, 35 aa, synthetic construct
  REGION 1..35: note = Artificially Synthesized Sequence
RQSGVPSRFSGSGSGTDFTLTISSLQPEDFATYYC

SEQ ID NO: 44 - protein, 10 aa, synthetic construct
  REGION 1..10: note = Artificially Synthesized Sequence
FGQGTKLEIK

SEQ ID NO: 45 - protein, 18 aa, synthetic construct
  REGION 1..18: note = Artificially Synthesized Sequence
LAWYQQKPGQAPRSLIYA

SEQ ID NO: 46 - protein, 35 aa, synthetic construct
  REGION 1..35: note = Artificially Synthesized Sequence
LQSGIPARFSGSGSGTDFTLTISSLEPEDFAVYYC

SEQ ID NO: 47 - protein, 18 aa, synthetic construct
  REGION 1..18: note = Artificially Synthesized Sequence
LAWYQQKPGQAPRSLIYS

SEQ ID NO: 48 - protein, 35 aa, synthetic construct
  REGION 1..35: note = Artificially Synthesized Sequence
RQSGIPARFSGSGSGTDFTLTISSLEPEDFAVYYC

SEQ ID NO: 49 - protein, 449 aa, synthetic construct
  REGION 1..449: note = Artificially Synthesized Sequence
EVQLVQSGAEVKKPGESLKISCQSSGYSFTTYWIGWVRQMPGQGLEWIGIMSPVDSDIRYNPMFRGQVTMSVDKSSSTAYLQWSSLKASDTAMYYCARRRPGQGYFDFWGQGTMVTVSSASTKGPSVFPLAPSSKSTSGGTAALGCLVKDYFPEPVTVSWNSGALTSGVHTFPAVLQSSGLYSLSSVVTVPSSSLGTQTYICNVNHKPSNTKVDKKVEPKSCDKTHTCPPCPAPELLGGPSVFLFPPKPKDTLMISRTPEVTCVVVDVSHEDPEVKFNWYVDGVEVHNAKTKPREEQYNSTYRVVSVLTVLHQDWLNGKEYKCKVSNKALPAPIEKTISKAKGQPREPQVYTLPPSREEMTKNQVSLTCLVKGFYPSDIAVEWESNGQPENNYKTTPPVLDSDGSFFLYSKLTVDKSRWQQGNVFSCSVMHEALHNHYTQKSLSLSPGK

SEQ ID NO: 50 - protein, 214 aa, synthetic construct
  REGION 1..214: note = Artificially Synthesized Sequence
DIQMTQSPSSLSASVGDRVTITCKASQNVGSWLAWYQQKPGKAPKSLIYSASSRQSGVPSRFSGSGSGTDFTLTISSLQPEDFATYYCQQYDIYPFTFGQGTKLEIKRTVAAPSVFIFPPSDEQLKSGTASVVCLLNNFYPREAKVQWKVDNALQSGNSQESVTEQDSKDSTYSLSSTLTLSKADYEKHKVYACEVTHQGLSSPVTKSFNRGEC

SEQ ID NO: 51 - protein, 214 aa, synthetic construct
  REGION 1..214: note = Artificially Synthesized Sequence
EIVLTQSPATLSASPGERATISCRASQSVGSWLAWYQQKPGQAPRSLIYAASNLQSGIPARFSGSGSGTDFTLTISSLEPEDFAVYYCQQYNIYPYTFGQGTRLEIKRTVAAPSVFIFPPSDEQLKSGTASVVCLLNNFYPREAKVQWKVDNALQSGNSQESVTEQDSKDSTYSLSSTLTLSKADYEKHKVYACEVTHQGLSSPVTKSFNRGEC

SEQ ID NO: 52 - protein, 214 aa, synthetic construct
  REGION 1..214: note = Artificially Synthesized Sequence
EIVLTQSPATLSASPGERATISCRASQSVSSWLAWYQQKPGQAPRSLIYSASNLQSGIPARFSGSGSGTDFTLTISSLEPEDFAVYYCQQYNIYPYTFGQGTRLEIKRTVAAPSVFIFPPSDEQLKSGTASVVCLLNNFYPREAKVQWKVDNALQSGNSQESVTEQDSKDSTYSLSSTLTLSKADYEKHKVYACEVTHQGLSSPVTKSFNRGEC

SEQ ID NO: 53 - protein, 214 aa, synthetic construct
  REGION 1..214: note = Artificially Synthesized Sequence
EIVLTQSPATLSASPGERATISCRASQSVSSWLAWYQQKPGQAPRSLIYAASNRQSGIPARFSGSGSGTDFTLTISSLEPEDFAVYYCQQYNIYPYTFGQGTRLEIKRTVAAPSVFIFPPSDEQLKSGTASVVCLLNNFYPREAKVQWKVDNALQSGNSQESVTEQDSKDSTYSLSSTLTLSKADYEKHKVYACEVTHQGLSSPVTKSFNRGEC

SEQ ID NO: 54 - protein, 214 aa, synthetic construct
  REGION 1..214: note = Artificially Synthesized Sequence
EIVLTQSPATLSASPGERATISCRASQSVSSWLAWYQQKPGQAPRSLIYAASNLQSGIPARFSGSGSGTDFTLTISSLEPEDFAVYYCQQYNIYPFTFGQGTRLEIKRTVAAPSVFIFPPSDEQLKSGTASVVCLLNNFYPREAKVQWKVDNALQSGNSQESVTEQDSKDSTYSLSSTLTLSKADYEKHKVYACEVTHQGLSSPVTKSFNRGEC